European Patent Application EP 4 428 236 A1, published September 11, 2024. Title: Antisense Oligonucleotide. Applicant: AUTOTELIC Bio Inc. The sequence listing filed with the application follows.

SEQUENCE LISTING (4 sequences)

SEQ ID NO: 1 - DNA, 20 bp, Artificial Sequence
  Antisense Oligonucleotide
ggcggcatgtctattttgta

SEQ ID NO: 2 - DNA, 20 bp, Artificial Sequence
  Antisense Oligonucleotide
cggcatgtctattttgtaaa

SEQ ID NO: 3 - DNA, 20 bp, Artificial Sequence
  Antisense Oligonucleotide
gcggcatgtctattttgtaa

SEQ ID NO: 4 - DNA, 5952 bp, Homo sapiens
gatgttatctgctggcagcagaaggttcgctccgagcggagctccagaagctcctgacaagagaaagacagattgagatagagatagaaagagaaagagagaaagagacagcagagcgagagcgcaagtgaaagaggcaggggagggggatggagaatattagcctgacggtctagggagtcatccaggaacaaactgaggggctgcccggctgcagacaggaggagacagagaggatctattttagggtggcaagtgcctacctaccctaagcgagcaattccacgttggggagaagccagcagaggttgggaaagggtgggagtccaagggagcccctgcgcaaccccctcaggaataaaactccccagccagggtgtcgcaagggctgccgttgtgatccgcagggggtgaacgcaaccgcgacggctgatcgtctgtggctgggttggcgtttggagcaagagaaggaggagcaggagaaggagggagctggaggctggaagcgtttgcaagcggcggcggcagcaacgtggagtaaccaagcgggtcagcgcgcgcccgccagggtgtaggccacggagcgcagctcccagagcaggatccgcgccgcctcagcagcctctgcggcccctgcggcacccgaccgagtaccgagcgccctgcgaagcgcaccctcctccccgcggtgcgctgggctcgcccccagcgcgcgcacacgcacacacacacacacacacacacacgcacgcacacacgtgtgcgcttctctgctccggagctgctgctgctcctgctctcagcgccgcagtggaaggcaggaccgaaccgctccttctttaaatatataaatttcagcccaggtcagcctcggcggcccccctcaccgcgctcccggcgcccctcccgtcagttcgccagctgccagccccgggaccttttcatctcttcccttttggccggaggagccgagttcagatccgccactccgcacccgagactgacacactgaactccacttcctcctcttaaatttatttctacttaatagccactcgtctctttttttccccatctcattgctccaagaatttttttcttcttactcgccaaagtcagggttccctctgcccgtcccgtattaatatttccacttttggaactactggccttttctttttaaaggaattcaagcaggatacgtttttctgttgggcattgactagattgtttgcaaaagtttcgcatcaaaaacaacaacaacaaaaaaccaaacaactctccttgatctatactttgagaattgttgatttcttttttttattctgacttttaaaaacaacttttttttccacttttttaaaaaatgcactactgtgtgctgagcgcttttctgatcctgcatctggtcacggtcgcgctcagcctgtctacctgcagcacactcgatatggaccagttcatgcgcaagaggatcgaggcgatccgcgggcagatcctgagcaagctgaagctcaccagtcccccagaagactatcctgagcccgaggaagtccccccggaggtgatttccatctacaacagcaccagggacttgctccaggagaaggcgagccggagggcggccgcctgcgagcgcgagaggagcgacgaagagtactacgccaaggaggtttacaaaatagacatgccgcccttcttcccctccgaaactgtctgcccagttgttacaacaccctctggctcagtgggcagcttgtgctccagacagtcccaggtgctctgtgggtaccttgatgccatcccgcccactttctacagaccctacttcagaattgttcgatttgacgtctcagcaatggagaagaatgcttccaatttggtgaaagcagagttcagagtctttcgtttgcagaacccaaaagccagagtgcctgaacaacggattgagctatatcagattctcaagtccaaagatttaacatctccaacccagcgctacatcgacagcaaagttgtgaaaacaagagcagaaggcgaatggctctccttcgatgtaactgatgctgttcatgaatggcttcaccataaagacaggaacctgggatttaaaataagcttacactgtccctgctgcacttttgtaccatctaataattacatcatcccaaataaaagtgaagaactagaagcaagatttgcaggtattgatggcacctccacatataccagtggtgatcagaaaactataaagtccactaggaaaaaaaacagtgggaagaccccacatctcctgctaatgttattgccctcctacagacttgagtcacaacagaccaaccggcggaagaagcgtgctttggatgcggcctattgctttagaaatgtgcaggataattgctgcctacgtccactttacattgatttcaagagggatctagggtggaaatggatacacgaacccaaagggtacaatgccaacttctgtgctggagcatgcccgtatttatggagttcagacactcagcacagcagggtcctgagcttatataataccataaatccagaagcatctgcttctccttgctgcgtgtcccaagatttagaacctctaaccattctctactacattggcaaaacacccaagattgaacagctttctaatatgattgtaaagtcttgcaaatgcagctaaaattcttggaaaagtggcaagaccaaaatgacaatgatgatgataatgatgatgacgacgacaacgatgatgcttgtaacaagaaaacataagagagccttggttcatcagtgttaaaaaatttttgaaaaggcggtactagttcagacactttggaagtttgtgttctgtttgttaaaactggcatctgacacaaaaaaagttgaaggccttattctacatttcacctactttgtaagtgagagagacaagaagcaaattttttttaaagaaaaaaataaacactggaagaatttattagtgttaattatgtgaacaacgacaacaacaacaacaacaacaaacaggaaaatcccattaagtggagttgctgtacgtaccgttcctatcccgcgcctcacttgatttttctgtattgctatgcaataggcacccttcccattcttactcttagagttaacagtgagttatttattgtgtgttactatataatgaacgtttcattgcccttggaaaataaaacaggtgtataaagtggagaccaaatactttgccagaaactcatggatggcttaaggaacttgaactcaaacgagccagaaaaaaagaggtcatattaatgggatgaaaacccaagtgagttattatatgaccgagaaagtctgcattaagataaagaccctgaaaacacatgttatgtatcagctgcctaaggaagcttcttgtaaggtccaaaaactaaaaagactgttaataaaagaaactttcagtcagaataagtctgtaagtttttttttttctttttaattgtaaatggttctttgtcagtttagtaaaccagtgaaatgttgaaatgttttgacatgtactggtcaaacttcagaccttaaaatattgctgtatagctatgctataggttttttcctttgttttggtatatgtaaccatacctatattattaaaatagatggatatagaagccagcataattgaaaacacatctgcagatctcttttgcaaactattaaatcaaaacattaactactttatgtgtaatgtgtaaatttttaccatattttttatattctgtaataatgtcaactatgatttagattgacttaaatttgggctctttttaatgatcactcacaaatgtatgtttcttttagctggccagtacttttgagtaaagcccctatagtttgacttgcactacaaatgcattttttttttaataacatttgccctacttgtgctttgtgtttctttcattattatgacataagctacctgggtccacttgtcttttcttttttttgtttcacagaaaagatgggttcgagttcagtggtcttcatcttccaagcatcattactaaccaagtcagacgttaacaaatttttatgttaggaaaaggaggaatgttatagatacatagaaaattgaagtaaaatgttttcattttagcaaggatttagggttctaactaaaactcagaatctttattgagttaagaaaagtttctctaccttggtttaatcaatatttttgtaaaatcctattgttattacaaagaggacacttcataggaaacatctttttctttagtcaggtttttaatattcagggggaaattgaaagatatatattttagtcgatttttcaaaaggggaaaaaagtccaggtcagcataagtcattttgtgtatttcactgaagttataaggtttttataaatgttctttgaaggggaaaaggcacaagccaatttttcctatgatcaaaaaattctttctttcctctgagtgagagttatctatatctgaggctaaagtttaccttgctttaataaataatttgccacatcattgcagaagaggtatcctcatgctggggttaatagaatatgtcagtttatcacttgtcgcttatttagctttaaaataaaaattaataggcaaagcaatggaatatttgcagtttcacctaaagagcagcataaggaggcgggaatccaaagtgaagttgtttgatatggtctacttcttttttggaatttcctgaccattaattaaagaattggatttgcaagtttgaaaactggaaaagcaagagatgggatgccataatagtaaacagcccttgtgttggatgtaacccaatcccagatttgagtgtgtgttgattatttttttgtcttccacttttctattatgtgtaaatcacttttatttctgcagacattttcctctcagataggatgacattttgttttgtattattttgtctttcctcatgaatgcactgataatattttaaatgctctattttaagatctcttgaatctgttttttttttttttaatttgggggttctgtaaggtctttatttcccataagtaaatattgccatgggaggggggtggaggtggcaaggaaggggtgaagtgctagtatgcaagtgggcagcaattatttttgtgttaatcagcagtacaatttgatcgttggcatggttaaaaaatggaatataagattagctgttttgtattttgatgaccaattacgctgtattttaacacgatgtatgtctgtttttgtggtgctctagtggtaaataaattatttcgatgatatgtggatgtctttttcctatcagtaccatcatcgagtctagaaaacacctgtgatgcaataagactatctcaagctggaaaagtcataccacctttccgattgccctctgtgctttctcccttaaggacagtcacttcagaagtcatgctttaaagcacaagagtcaggccatatccatcaaggatagaagaaatccctgtgccgtctttttattcccttatttattgctatttggtaattgtttgagatttagtttccatccagcttgactgccgaccagaaaaaatgcagagagatgtttgcaccatgctttggctttctggttctatgttctgccaacgccagggccaaaagaactggtctagacagtatcccctgtagccccataacttggatagttgctgagccagccagatataacaagagccacgtgctttctggggttggttgtttgggatcagctacttgcctgtcagtttcactggtaccactgcaccacaaacaaaaaaacccaccctatttcctccaatttttttggctgctacctacaagaccagactcctcaaacgagttgccaatctcttaataaataggattaataaaaaaagtaattgtgactcaa